European Patent Specification EP 3 587 440 B1, published March 15, 2023. Title: 一种人PD-L1蛋白高亲和性肽及其应用. Applicant: 朱乃硕. The sequence listing filed with the application follows.

SEQUENCE LISTING (5 sequences)

SEQ ID NO: 1 - protein, 12 aa
VSVSHFQKVWVV

SEQ ID NO: 2 - DNA, 45 bp
gtgagtgtgtcgcattttcagaaggtttgggttgtgggtggaggt

SEQ ID NO: 3 - protein, 12 aa
HESWLPAYVLGS

SEQ ID NO: 4 - protein, 12 aa
HTSWILYGETGW

SEQ ID NO: 5 - protein, 40 aa
VSVSHFQKVWVVDMHESWLPAYVLGSDMHTSWILYGETGW